European Patent Application EP 4 349 846 A1, published April 10, 2024. Title: PHOSOPHOROTHIOATE AND BORANOPHOSPHATE-INCLUDING CHIMERIC NUCLEIC ACID OLIGOMER AND METHOD FOR PRODUCING SAME. Applicant: TOKYO UNIVERSITY OF SCIENCE FOUNDATION. The sequence listing filed with the application follows.

SEQUENCE LISTING (7 sequences)

SEQ ID NO: 1 - DNA, 12 bp, Artificial Sequence
  Sequence for demonstration
cagtcagtcagt

SEQ ID NO: 2 - RNA, 12 nt, Homo sapiens
gaauaccaaugc

SEQ ID NO: 3 - DNA, 12 bp, Artificial Sequence
  Antisence oligomer for apoB (PB/PS/PO chimera)
gcattggtattc

SEQ ID NO: 4 - DNA, 12 bp, Artificial Sequence
  Antisence oligomer for apoB (PB/PS/PO-gapmer)
  DNA/RNA chimera
gcattggtauuc

SEQ ID NO: 5 - DNA, 12 bp, Artificial Sequence
  Antisence oligomer for apoB (PB/PS chimera)
gcattggtattc

SEQ ID NO: 6 - DNA, 12 bp, Artificial Sequence
  Antisence oligomer for apoB (PB/PS-LNA-gapmer)
  DNA/RNA chimera
gcattggtattc

SEQ ID NO: 7 - DNA, 12 bp, Artificial Sequence
  Antisence oligomer for apoB (PB/PS/PO-mixmer)
  DNA/RNA chimera
gcattggtattc